European Patent Specification EP 4 448 786 B1, published February 4, 2026. Title: METHODS FOR METAL DIRECTED CLEAVAGE OF SURFACE-BOUND POLYNUCLEOTIDES. Applicant: Illumina Cambridge Limited. Application WO. The sequence listing filed with the application follows.

SEQUENCE LISTING (10 sequences)

SEQ ID NO: 1 - DNA, 29 bp, synthetic construct
  misc_feature 1..29: note = Synthetic Oligonucleotide
  source 1..29: mol_type = other DNA
  misc_feature 23: note = n = uracil
aatgatacggcgaccaccgaganctacac

SEQ ID NO: 2 - DNA, 24 bp, synthetic construct
  misc_feature 1..24: note = Synthetic Oligonucleotide
  misc_feature 22: note = n = 8-oxo-guanine
  source 1..24: mol_type = other DNA
caagcagaagacggcatacganat

SEQ ID NO: 3 - DNA, 39 bp, synthetic construct
  misc_feature 1..39: note = Synthetic Oligonucleotide
  misc_feature 1: note = 5'-alkyne
  source 1..39: mol_type = other DNA
  misc_feature 33: note = n = uracil
ttttttttttaatgatacggcgaccaccgaganctacac

SEQ ID NO: 4 - DNA, 34 bp, synthetic construct
  misc_feature 1..34: note = Synthetic Oligonucleotide
  misc_feature 32: note = n = 8-oxo-guanine
  misc_feature 1: note = 5'-alkyne
  source 1..34: mol_type = other DNA
ttttttttttcaagcagaagacggcatacganat

SEQ ID NO: 5 - DNA, 20 bp, synthetic construct
  misc_feature 1..20: note = Synthetic Oligonucleotide
  source 1..20: mol_type = other DNA
aatgatacggcgaccaccga

SEQ ID NO: 6 - DNA, 21 bp, synthetic construct
  misc_feature 1..21: note = Synthetic Oligonucleotide
  source 1..21: mol_type = other DNA
caagcagaagacggcatacga

SEQ ID NO: 7 - DNA, 29 bp, synthetic construct
  misc_feature 1..29: note = Synthetic Oligonucleotide
  misc_feature 23: note = n = vinyl substituted T nucleoside
  source 1..29: mol_type = other DNA
aatgatacggcgaccaccgaganctacac

SEQ ID NO: 8 - DNA, 27 bp, synthetic construct
  misc_feature 1..27: note = Synthetic Oligonucleotide
  misc_feature 1..3: note = diol linker subject to chemical cleavage
  source 1..27: mol_type = other DNA
yyycaagcagaagacggcatacgagat

SEQ ID NO: 9 - DNA, 35 bp, synthetic construct
  misc_feature 1..35: note = Synthetic Oligonucleotide
  misc_feature 29: note = n = a vinyl substituted T nucleoside
  misc_feature 1: note = 5'-alkyne
  source 1..35: mol_type = other DNA
ttttttaatgatacggcgaccaccgaganctacac

SEQ ID NO: 10 - DNA, 33 bp, synthetic construct
  misc_feature 1..33: note = Synthetic Oligonucleotide
  misc_feature 7..9: note = diol linker subject to chemical cleavage
  misc_feature 1: note = 5'-alkyne
  source 1..33: mol_type = other DNA
ttttttyyycaagcagaagacggcatacgagat